European Patent Application EP 4 682 161 A1, published January 21, 2026. Title: tkt基因突变体及其在制备L-赖氨酸中的应用. Applicant: 黑龙江伊品生物科技有限公司. Application CN. The sequence listing filed with the application follows.

SEQUENCE LISTING (49 sequences)

SEQ ID NO: 1 - DNA, 2103 bp, synthetic construct
  source 1..2103: mol_type = other DNA
ttgaccaccttgacgctgtcacctgaacttcaggcgctcactgtacgcaattacccctctgattggtccgatgtggacaccaaggctgtagacactgttcgtgtcctcgctgcagacgctgtagaaaactgtggctccggccacccaggcaccgcaatgagcctggctccccttgcatacaccttgtaccagcgggttatgaacgtagatccacaggacaccaactgggcaggccgtgaccgcttcgttctttcttgtggccactcctctttgacccagtacatccagctttacttgggtggattcggccttgagatggatgacctgaaggctctgcgcacctgggattccttgaccccaggacaccctgagtaccgccacaccaagggcgttgagatcaccactggccctcttggccagggtcttgcatctgcagttggtatggccatggctgctcgtcgtgagcgtggcctattcgacccaaccgctgctgagggcgaatccccattcgaccaccacatctacgtcattgcttctgatggtgacctgcaggaaggtgtcacctctgaggcatcctccatcgctggcacccagcagctgggcaacctcatcgtgttctgggatgacaaccgcatctccatcgaagacaacactgagatcgctttcaacgaggacgttgttgctcgttacaaggcttacggctggcagaccattgaggttgaggctggcgaggacgttgcagcaatcgaagctgcagtggctgaggctaagaaggacaccaagcgacctaccttcatccgcgttcgcaccatcatcggcttcccagctccaactatgatgaacaccggtgctgtgcacggtgctgctcttggcgcagctgaggttgcagcaaccaagactgagcttggattcgatcctgaggctcacttcgcgatcgacgatgaggttatcgctcacacccgctccctcgcagagcgcgctgcacagaagaaggctgcatggcaggtcaagttcgatgagtgggcagctgccaaccctgagaacaaggctctgttcgatcgcctgaactcccgtgagcttccagcgggctacgctgacgagctcccaacatgggatgcagatgagaagggcgtcgcaactcgtaaggcttccgaggctgcacttcaggcactgggcaagacccttcctgagctgtggggcggttccgctgacctcgcaggttccaacaacaccgtgatcaagggctccccttccttcggccctgagtccatctccaccgagacctggtctgctgagccttacggccgtaacctgcacttcggtatccgtgagcacgctatgggatccatcctcaacggcatttccctccacggtggcacccgcccatacggcggaaccttcctcatcttctccgactacatgcgtcctgcagttcgtcttgcagctctcatggagaccgacgcttactacgtctggacccacgactccatcggtctgggcgaagatggcccaacccaccagcctgttgaaaccttggctgcactgcgcgccatcccaggtctgtccgtcctgcgtcctgcagatgcgaacgagaccgcccaggcttgggctgcagcacttgagtacaaggaaggccctaagggtcttgcactgacccgccagaacgttcctgttctggaaggcaccaaggagaaggctgctgaaggcgttcgccgcggtggctacgtcctggttgagggttccaaggaaaccccagatgtgatcctcatgggctccggctccgaggttcagcttgcagttaacgctgcgaaggctctggaagctgagggcgttgcagctcgcgttgtttccgttccttgcatggattggttccaggagcaggacgcagagtacatcgagtccgttctgcctgcagctgtgaccgctcgtgtgtctgttgaagctggcatcgcaatgccttggtaccgcttcttgggcacccagggccgtgctgtctcccttgagcacttcggtgcttctgcggattaccagaccctgtttgagaagttcggcatcaccaccgatgcagtcgtggcagcggccaaggactccattaacggttaa

SEQ ID NO: 2 - protein, 700 aa, synthetic construct
MTTLTLSPELQALTVRNYPSDWSDVDTKAVDTVRVLAADAVENCGSGHPGTAMSLAPLAYTLYQRVMNVDPQDTNWAGRDRFVLSCGHSSLTQYIQLYLGGFGLEMDDLKALRTWDSLTPGHPEYRHTKGVEITTGPLGQGLASAVGMAMAARRERGLFDPTAAEGESPFDHHIYVIASDGDLQEGVTSEASSIAGTQQLGNLIVFWDDNRISIEDNTEIAFNEDVVARYKAYGWQTIEVEAGEDVAAIEAAVAEAKKDTKRPTFIRVRTIIGFPAPTMMNTGAVHGAALGAAEVAATKTELGFDPEAHFAIDDEVIAHTRSLAERAAQKKAAWQVKFDEWAAANPENKALFDRLNSRELPAGYADELPTWDADEKGVATRKASEAALQALGKTLPELWGGSADLAGSNNTVIKGSPSFGPESISTETWSAEPYGRNLHFGIREHAMGSILNGISLHGGTRPYGGTFLIFSDYMRPAVRLAALMETDAYYVWTHDSIGLGEDGPTHQPVETLAALRAIPGLSVLRPADANETAQAWAAALEYKEGPKGLALTRQNVPVLEGTKEKAAEGVRRGGYVLVEGSKETPDVILMGSGSEVQLAVNAAKALEAEGVAARVVSVPCMDWFQEQDAEYIESVLPAAVTARVSVEAGIAMPWYRFLGTQGRAVSLEHFGASADYQTLFEKFGITTDAVVAAAKDSING

SEQ ID NO: 3 - DNA, 2103 bp, synthetic construct
  source 1..2103: mol_type = other DNA
ttgaccaccttgacgctgtcacctgaacttcaggcgctcactgtacgcaattacccctctgattggtccgatgtggacaccaaggctgtagacactgttcgtgtcctcgctgcagacgctgtagaaaactgtggctccggccacccaggcaccgcaatgagcctggctccccttgcatacaccttgtaccagcgggttatgaacgtagatccacaggacaccaactgggcaggccgtgaccgcttcgttctttcttgtggccactcctctttgacccagtacatccagctttacttgggtggattcggccttgagatggatgacctgaaggctctgcgcacctgggattccttgaccccaggacaccctgagtaccgccacaccaagggcgttgagatcaccactggccctcttggccagggtcttgcatctgcagttggtatggccatggctgctcgtcgtgagcgtggcctattcgacccaaccgctgctgagggcgaatccccattcgaccaccacatctacgtcattgcttctgatggtgacctgcaggaaggtgtcacctctgaggcatcctccatcgctggcacccagcagctgggcaacctcatcgtgttctgggatgacaaccgcatctccatcgaagacaacactgagatcgctttcaacgaggacgttgttgctcgttacaaggcttacggctggcagaccattgaggttgaggctggcgaggacgttgcagcaatcgaagctgcagtggctgaggctaagaaggacaccaagcgacctaccttcatccgcgttcgcaccatcatcggcttcccagctccaactatgatgaacaccggtgctgtgcacggtgctgctcttggcgcagctgaggttgcagcaaccaagactgagcttggattcgatcctgaggctcacttcgcgatcgacgatgaggttatcgctcacacccgctccctcgcagagcgcactgcacagaagaaggctgcatggcaggtcaagttcgatgagtgggcagctgccaaccctgagaacaaggctctgttcgatcgcctgaactcccgtgagcttccagcgggctacgctgacgagctcccaacatgggatgcagatgagaagggcgtcgcaactcgtaaggcttccgaggctgcacttcaggcactgggcaagacccttcctgagctgtggggcggttccgctgacctcgcaggttccaacaacaccgtgatcaagggctccccttccttcggccctgagtccatctccaccgagacctggtctgctgagccttacggccgtaacctgcacttcggtatccgtgagcacgctatgggatccatcctcaacggcatttccctccacggtggcacccgcccatacggcggaaccttcctcatcttctccgactacatgcgtcctgcagttcgtcttgcagctctcatggagaccgacgcttactacgtctggacccacgactccatcggtctgggcgaagatggcccaacccaccagcctgttgaaaccttggctgcactgcgcgccatcccaggtctgtccgtcctgcgtcctgcagatgcgaacgagaccgcccaggcttgggctgcagcacttgagtacaaggaaggccctaagggtcttgcactgacccgccagaacgttcctgttctggaaggcaccaaggagaaggctgctgaaggcgttcgccgcggtggctacgtcctggttgagggttccaaggaaaccccagatgtgatcctcatgggctccggctccgaggttcagcttgcagttaacgctgcgaaggctctggaagctgagggcgttgcagctcgcgttgtttccgttccttgcatggattggttccaggagcaggacgcagagtacatcgagtccgttctgcctgcagctgtgaccgctcgtgtgtctgttgaagctggcatcgcaatgccttggtaccgcttcttgggcacccagggccgtgctgtctcccttgagcacttcggtgcttctgcggattaccagaccctgtttgagaagttcggcatcaccaccgatgcagtcgtggcagcggccaaggactccattaacggttaa

SEQ ID NO: 4 - protein, 700 aa, synthetic construct
MTTLTLSPELQALTVRNYPSDWSDVDTKAVDTVRVLAADAVENCGSGHPGTAMSLAPLAYTLYQRVMNVDPQDTNWAGRDRFVLSCGHSSLTQYIQLYLGGFGLEMDDLKALRTWDSLTPGHPEYRHTKGVEITTGPLGQGLASAVGMAMAARRERGLFDPTAAEGESPFDHHIYVIASDGDLQEGVTSEASSIAGTQQLGNLIVFWDDNRISIEDNTEIAFNEDVVARYKAYGWQTIEVEAGEDVAAIEAAVAEAKKDTKRPTFIRVRTIIGFPAPTMMNTGAVHGAALGAAEVAATKTELGFDPEAHFAIDDEVIAHTRSLAERTAQKKAAWQVKFDEWAAANPENKALFDRLNSRELPAGYADELPTWDADEKGVATRKASEAALQALGKTLPELWGGSADLAGSNNTVIKGSPSFGPESISTETWSAEPYGRNLHFGIREHAMGSILNGISLHGGTRPYGGTFLIFSDYMRPAVRLAALMETDAYYVWTHDSIGLGEDGPTHQPVETLAALRAIPGLSVLRPADANETAQAWAAALEYKEGPKGLALTRQNVPVLEGTKEKAAEGVRRGGYVLVEGSKETPDVILMGSGSEVQLAVNAAKALEAEGVAARVVSVPCMDWFQEQDAEYIESVLPAAVTARVSVEAGIAMPWYRFLGTQGRAVSLEHFGASADYQTLFEKFGITTDAVVAAAKDSING

SEQ ID NO: 5 - DNA, 2103 bp, synthetic construct
  source 1..2103: mol_type = other DNA
ttgaccaccttgacgctgtcacctgaacttcaggcgctcactgtacgcaattacccctctgattggtccgatgtggacaccaaggctgtagacactgttcgtgtcctcgctgcagacgctgtagaaaactgtggctccggccacccaggcaccgcaatgagcctggctccccttgcatacaccttgtaccagcgggttatgaacgtagatccacaggacaccaactgggcaggccgtgaccgcttcgttctttcttgtggccactcctctttgacccagtacatccagctttacttgggtggattcggccttgagatggatgacctgaaggctctgcgcacctgggattccttgaccccaggacaccctgagtaccgccacaccaagggcgttgagatcaccactggccctcttggccagggtcttgcatctgcagttggtatggccatggctgctcgtcgtgagcgtggcctattcgacccaaccgctgctgagggcgaatccccattcgaccaccacatctacgtcattgcttctgatggtgacctgcaggaaggtgtcacctctgaggcatcctccatcgctggcacccagcagctgggcaacctcatcgtgttctgggatgacaaccgcatctccatcgaagacaacactgagatcgctttcaacgaggacgttgttgctcgttacaaggcttacggctggcagaccattgaggttgaggctggcgaggacgttgcagcaatcgaagctgcagtggctgaggctaagaaggacaccaagcgacctaccttcatccgcgttcgcaccatcatcggcttcccagctccaactatgatgaacaccggtgctgtgcacggtgctgctcttggcgcagctgaggttgcagcaaccaagactgagcttggattcgatcctgaggctcacttcgcgatcgacgatgaggttatcgctcacacccgctccctcgcagagcgctctgcacagaagaaggctgcatggcaggtcaagttcgatgagtgggcagctgccaaccctgagaacaaggctctgttcgatcgcctgaactcccgtgagcttccagcgggctacgctgacgagctcccaacatgggatgcagatgagaagggcgtcgcaactcgtaaggcttccgaggctgcacttcaggcactgggcaagacccttcctgagctgtggggcggttccgctgacctcgcaggttccaacaacaccgtgatcaagggctccccttccttcggccctgagtccatctccaccgagacctggtctgctgagccttacggccgtaacctgcacttcggtatccgtgagcacgctatgggatccatcctcaacggcatttccctccacggtggcacccgcccatacggcggaaccttcctcatcttctccgactacatgcgtcctgcagttcgtcttgcagctctcatggagaccgacgcttactacgtctggacccacgactccatcggtctgggcgaagatggcccaacccaccagcctgttgaaaccttggctgcactgcgcgccatcccaggtctgtccgtcctgcgtcctgcagatgcgaacgagaccgcccaggcttgggctgcagcacttgagtacaaggaaggccctaagggtcttgcactgacccgccagaacgttcctgttctggaaggcaccaaggagaaggctgctgaaggcgttcgccgcggtggctacgtcctggttgagggttccaaggaaaccccagatgtgatcctcatgggctccggctccgaggttcagcttgcagttaacgctgcgaaggctctggaagctgagggcgttgcagctcgcgttgtttccgttccttgcatggattggttccaggagcaggacgcagagtacatcgagtccgttctgcctgcagctgtgaccgctcgtgtgtctgttgaagctggcatcgcaatgccttggtaccgcttcttgggcacccagggccgtgctgtctcccttgagcacttcggtgcttctgcggattaccagaccctgtttgagaagttcggcatcaccaccgatgcagtcgtggcagcggccaaggactccattaacggttaa

SEQ ID NO: 6 - protein, 700 aa, synthetic construct
MTTLTLSPELQALTVRNYPSDWSDVDTKAVDTVRVLAADAVENCGSGHPGTAMSLAPLAYTLYQRVMNVDPQDTNWAGRDRFVLSCGHSSLTQYIQLYLGGFGLEMDDLKALRTWDSLTPGHPEYRHTKGVEITTGPLGQGLASAVGMAMAARRERGLFDPTAAEGESPFDHHIYVIASDGDLQEGVTSEASSIAGTQQLGNLIVFWDDNRISIEDNTEIAFNEDVVARYKAYGWQTIEVEAGEDVAAIEAAVAEAKKDTKRPTFIRVRTIIGFPAPTMMNTGAVHGAALGAAEVAATKTELGFDPEAHFAIDDEVIAHTRSLAERSAQKKAAWQVKFDEWAAANPENKALFDRLNSRELPAGYADELPTWDADEKGVATRKASEAALQALGKTLPELWGGSADLAGSNNTVIKGSPSFGPESISTETWSAEPYGRNLHFGIREHAMGSILNGISLHGGTRPYGGTFLIFSDYMRPAVRLAALMETDAYYVWTHDSIGLGEDGPTHQPVETLAALRAIPGLSVLRPADANETAQAWAAALEYKEGPKGLALTRQNVPVLEGTKEKAAEGVRRGGYVLVEGSKETPDVILMGSGSEVQLAVNAAKALEAEGVAARVVSVPCMDWFQEQDAEYIESVLPAAVTARVSVEAGIAMPWYRFLGTQGRAVSLEHFGASADYQTLFEKFGITTDAVVAAAKDSING

SEQ ID NO: 7 - DNA, 2103 bp, synthetic construct
  source 1..2103: mol_type = other DNA
ttgaccaccttgacgctgtcacctgaacttcaggcgctcactgtacgcaattacccctctgattggtccgatgtggacaccaaggctgtagacactgttcgtgtcctcgctgcagacgctgtagaaaactgtggctccggccacccaggcaccgcaatgagcctggctccccttgcatacaccttgtaccagcgggttatgaacgtagatccacaggacaccaactgggcaggccgtgaccgcttcgttctttcttgtggccactcctctttgacccagtacatccagctttacttgggtggattcggccttgagatggatgacctgaaggctctgcgcacctgggattccttgaccccaggacaccctgagtaccgccacaccaagggcgttgagatcaccactggccctcttggccagggtcttgcatctgcagttggtatggccatggctgctcgtcgtgagcgtggcctattcgacccaaccgctgctgagggcgaatccccattcgaccaccacatctacgtcattgcttctgatggtgacctgcaggaaggtgtcacctctgaggcatcctccatcgctggcacccagcagctgggcaacctcatcgtgttctgggatgacaaccgcatctccatcgaagacaacactgagatcgctttcaacgaggacgttgttgctcgttacaaggcttacggctggcagaccattgaggttgaggctggcgaggacgttgcagcaatcgaagctgcagtggctgaggctaagaaggacaccaagcgacctaccttcatccgcgttcgcaccatcatcggcttcccagctccaactatgatgaacaccggtgctgtgcacggtgctgctcttggcgcagctgaggttgcagcaaccaagactgagcttggattcgatcctgaggctcacttcgcgatcgacgatgaggttatcgctcacacccgctccctcgcagagcgctgtgcacagaagaaggctgcatggcaggtcaagttcgatgagtgggcagctgccaaccctgagaacaaggctctgttcgatcgcctgaactcccgtgagcttccagcgggctacgctgacgagctcccaacatgggatgcagatgagaagggcgtcgcaactcgtaaggcttccgaggctgcacttcaggcactgggcaagacccttcctgagctgtggggcggttccgctgacctcgcaggttccaacaacaccgtgatcaagggctccccttccttcggccctgagtccatctccaccgagacctggtctgctgagccttacggccgtaacctgcacttcggtatccgtgagcacgctatgggatccatcctcaacggcatttccctccacggtggcacccgcccatacggcggaaccttcctcatcttctccgactacatgcgtcctgcagttcgtcttgcagctctcatggagaccgacgcttactacgtctggacccacgactccatcggtctgggcgaagatggcccaacccaccagcctgttgaaaccttggctgcactgcgcgccatcccaggtctgtccgtcctgcgtcctgcagatgcgaacgagaccgcccaggcttgggctgcagcacttgagtacaaggaaggccctaagggtcttgcactgacccgccagaacgttcctgttctggaaggcaccaaggagaaggctgctgaaggcgttcgccgcggtggctacgtcctggttgagggttccaaggaaaccccagatgtgatcctcatgggctccggctccgaggttcagcttgcagttaacgctgcgaaggctctggaagctgagggcgttgcagctcgcgttgtttccgttccttgcatggattggttccaggagcaggacgcagagtacatcgagtccgttctgcctgcagctgtgaccgctcgtgtgtctgttgaagctggcatcgcaatgccttggtaccgcttcttgggcacccagggccgtgctgtctcccttgagcacttcggtgcttctgcggattaccagaccctgtttgagaagttcggcatcaccaccgatgcagtcgtggcagcggccaaggactccattaacggttaa

SEQ ID NO: 8 - protein, 700 aa, synthetic construct
MTTLTLSPELQALTVRNYPSDWSDVDTKAVDTVRVLAADAVENCGSGHPGTAMSLAPLAYTLYQRVMNVDPQDTNWAGRDRFVLSCGHSSLTQYIQLYLGGFGLEMDDLKALRTWDSLTPGHPEYRHTKGVEITTGPLGQGLASAVGMAMAARRERGLFDPTAAEGESPFDHHIYVIASDGDLQEGVTSEASSIAGTQQLGNLIVFWDDNRISIEDNTEIAFNEDVVARYKAYGWQTIEVEAGEDVAAIEAAVAEAKKDTKRPTFIRVRTIIGFPAPTMMNTGAVHGAALGAAEVAATKTELGFDPEAHFAIDDEVIAHTRSLAERCAQKKAAWQVKFDEWAAANPENKALFDRLNSRELPAGYADELPTWDADEKGVATRKASEAALQALGKTLPELWGGSADLAGSNNTVIKGSPSFGPESISTETWSAEPYGRNLHFGIREHAMGSILNGISLHGGTRPYGGTFLIFSDYMRPAVRLAALMETDAYYVWTHDSIGLGEDGPTHQPVETLAALRAIPGLSVLRPADANETAQAWAAALEYKEGPKGLALTRQNVPVLEGTKEKAAEGVRRGGYVLVEGSKETPDVILMGSGSEVQLAVNAAKALEAEGVAARVVSVPCMDWFQEQDAEYIESVLPAAVTARVSVEAGIAMPWYRFLGTQGRAVSLEHFGASADYQTLFEKFGITTDAVVAAAKDSING

SEQ ID NO: 9 - DNA, 2103 bp, synthetic construct
  source 1..2103: mol_type = other DNA
ttgaccaccttgacgctgtcacctgaacttcaggcgctcactgtacgcaattacccctctgattggtccgatgtggacaccaaggctgtagacactgttcgtgtcctcgctgcagacgctgtagaaaactgtggctccggccacccaggcaccgcaatgagcctggctccccttgcatacaccttgtaccagcgggttatgaacgtagatccacaggacaccaactgggcaggccgtgaccgcttcgttctttcttgtggccactcctctttgacccagtacatccagctttacttgggtggattcggccttgagatggatgacctgaaggctctgcgcacctgggattccttgaccccaggacaccctgagtaccgccacaccaagggcgttgagatcaccactggccctcttggccagggtcttgcatctgcagttggtatggccatggctgctcgtcgtgagcgtggcctattcgacccaaccgctgctgagggcgaatccccattcgaccaccacatctacgtcattgcttctgatggtgacctgcaggaaggtgtcacctctgaggcatcctccatcgctggcacccagcagctgggcaacctcatcgtgttctgggatgacaaccgcatctccatcgaagacaacactgagatcgctttcaacgaggacgttgttgctcgttacaaggcttacggctggcagaccattgaggttgaggctggcgaggacgttgcagcaatcgaagctgcagtggctgaggctaagaaggacaccaagcgacctaccttcatccgcgttcgcaccatcatcggcttcccagctccaactatgatgaacaccggtgctgtgcacggtgctgctcttggcgcagctgaggttgcagcaaccaagactgagcttggattcgatcctgaggctcacttcgcgatcgacgatgaggttatcgctcacacccgctccctcgcagagcgccctgcacagaagaaggctgcatggcaggtcaagttcgatgagtgggcagctgccaaccctgagaacaaggctctgttcgatcgcctgaactcccgtgagcttccagcgggctacgctgacgagctcccaacatgggatgcagatgagaagggcgtcgcaactcgtaaggcttccgaggctgcacttcaggcactgggcaagacccttcctgagctgtggggcggttccgctgacctcgcaggttccaacaacaccgtgatcaagggctccccttccttcggccctgagtccatctccaccgagacctggtctgctgagccttacggccgtaacctgcacttcggtatccgtgagcacgctatgggatccatcctcaacggcatttccctccacggtggcacccgcccatacggcggaaccttcctcatcttctccgactacatgcgtcctgcagttcgtcttgcagctctcatggagaccgacgcttactacgtctggacccacgactccatcggtctgggcgaagatggcccaacccaccagcctgttgaaaccttggctgcactgcgcgccatcccaggtctgtccgtcctgcgtcctgcagatgcgaacgagaccgcccaggcttgggctgcagcacttgagtacaaggaaggccctaagggtcttgcactgacccgccagaacgttcctgttctggaaggcaccaaggagaaggctgctgaaggcgttcgccgcggtggctacgtcctggttgagggttccaaggaaaccccagatgtgatcctcatgggctccggctccgaggttcagcttgcagttaacgctgcgaaggctctggaagctgagggcgttgcagctcgcgttgtttccgttccttgcatggattggttccaggagcaggacgcagagtacatcgagtccgttctgcctgcagctgtgaccgctcgtgtgtctgttgaagctggcatcgcaatgccttggtaccgcttcttgggcacccagggccgtgctgtctcccttgagcacttcggtgcttctgcggattaccagaccctgtttgagaagttcggcatcaccaccgatgcagtcgtggcagcggccaaggactccattaacggttaa

SEQ ID NO: 10 - protein, 700 aa, synthetic construct
MTTLTLSPELQALTVRNYPSDWSDVDTKAVDTVRVLAADAVENCGSGHPGTAMSLAPLAYTLYQRVMNVDPQDTNWAGRDRFVLSCGHSSLTQYIQLYLGGFGLEMDDLKALRTWDSLTPGHPEYRHTKGVEITTGPLGQGLASAVGMAMAARRERGLFDPTAAEGESPFDHHIYVIASDGDLQEGVTSEASSIAGTQQLGNLIVFWDDNRISIEDNTEIAFNEDVVARYKAYGWQTIEVEAGEDVAAIEAAVAEAKKDTKRPTFIRVRTIIGFPAPTMMNTGAVHGAALGAAEVAATKTELGFDPEAHFAIDDEVIAHTRSLAERPAQKKAAWQVKFDEWAAANPENKALFDRLNSRELPAGYADELPTWDADEKGVATRKASEAALQALGKTLPELWGGSADLAGSNNTVIKGSPSFGPESISTETWSAEPYGRNLHFGIREHAMGSILNGISLHGGTRPYGGTFLIFSDYMRPAVRLAALMETDAYYVWTHDSIGLGEDGPTHQPVETLAALRAIPGLSVLRPADANETAQAWAAALEYKEGPKGLALTRQNVPVLEGTKEKAAEGVRRGGYVLVEGSKETPDVILMGSGSEVQLAVNAAKALEAEGVAARVVSVPCMDWFQEQDAEYIESVLPAAVTARVSVEAGIAMPWYRFLGTQGRAVSLEHFGASADYQTLFEKFGITTDAVVAAAKDSING

SEQ ID NO: 11 - DNA, 2103 bp, synthetic construct
  source 1..2103: mol_type = other DNA
ttgaccaccttgacgctgtcacctgaacttcaggcgctcactgtacgcaattacccctctgattggtccgatgtggacaccaaggctgtagacactgttcgtgtcctcgctgcagacgctgtagaaaactgtggctccggccacccaggcaccgcaatgagcctggctccccttgcatacaccttgtaccagcgggttatgaacgtagatccacaggacaccaactgggcaggccgtgaccgcttcgttctttcttgtggccactcctctttgacccagtacatccagctttacttgggtggattcggccttgagatggatgacctgaaggctctgcgcacctgggattccttgaccccaggacaccctgagtaccgccacaccaagggcgttgagatcaccactggccctcttggccagggtcttgcatctgcagttggtatggccatggctgctcgtcgtgagcgtggcctattcgacccaaccgctgctgagggcgaatccccattcgaccaccacatctacgtcattgcttctgatggtgacctgcaggaaggtgtcacctctgaggcatcctccatcgctggcacccagcagctgggcaacctcatcgtgttctgggatgacaaccgcatctccatcgaagacaacactgagatcgctttcaacgaggacgttgttgctcgttacaaggcttacggctggcagaccattgaggttgaggctggcgaggacgttgcagcaatcgaagctgcagtggctgaggctaagaaggacaccaagcgacctaccttcatccgcgttcgcaccatcatcggcttcccagctccaactatgatgaacaccggtgctgtgcacggtgctgctcttggcgcagctgaggttgcagcaaccaagactgagcttggattcgatcctgaggctcacttcgcgatcgacgatgaggttatcgctcacacccgctccctcgcagagcgcaatgcacagaagaaggctgcatggcaggtcaagttcgatgagtgggcagctgccaaccctgagaacaaggctctgttcgatcgcctgaactcccgtgagcttccagcgggctacgctgacgagctcccaacatgggatgcagatgagaagggcgtcgcaactcgtaaggcttccgaggctgcacttcaggcactgggcaagacccttcctgagctgtggggcggttccgctgacctcgcaggttccaacaacaccgtgatcaagggctccccttccttcggccctgagtccatctccaccgagacctggtctgctgagccttacggccgtaacctgcacttcggtatccgtgagcacgctatgggatccatcctcaacggcatttccctccacggtggcacccgcccatacggcggaaccttcctcatcttctccgactacatgcgtcctgcagttcgtcttgcagctctcatggagaccgacgcttactacgtctggacccacgactccatcggtctgggcgaagatggcccaacccaccagcctgttgaaaccttggctgcactgcgcgccatcccaggtctgtccgtcctgcgtcctgcagatgcgaacgagaccgcccaggcttgggctgcagcacttgagtacaaggaaggccctaagggtcttgcactgacccgccagaacgttcctgttctggaaggcaccaaggagaaggctgctgaaggcgttcgccgcggtggctacgtcctggttgagggttccaaggaaaccccagatgtgatcctcatgggctccggctccgaggttcagcttgcagttaacgctgcgaaggctctggaagctgagggcgttgcagctcgcgttgtttccgttccttgcatggattggttccaggagcaggacgcagagtacatcgagtccgttctgcctgcagctgtgaccgctcgtgtgtctgttgaagctggcatcgcaatgccttggtaccgcttcttgggcacccagggccgtgctgtctcccttgagcacttcggtgcttctgcggattaccagaccctgtttgagaagttcggcatcaccaccgatgcagtcgtggcagcggccaaggactccattaacggttaa

SEQ ID NO: 12 - protein, 700 aa, synthetic construct
MTTLTLSPELQALTVRNYPSDWSDVDTKAVDTVRVLAADAVENCGSGHPGTAMSLAPLAYTLYQRVMNVDPQDTNWAGRDRFVLSCGHSSLTQYIQLYLGGFGLEMDDLKALRTWDSLTPGHPEYRHTKGVEITTGPLGQGLASAVGMAMAARRERGLFDPTAAEGESPFDHHIYVIASDGDLQEGVTSEASSIAGTQQLGNLIVFWDDNRISIEDNTEIAFNEDVVARYKAYGWQTIEVEAGEDVAAIEAAVAEAKKDTKRPTFIRVRTIIGFPAPTMMNTGAVHGAALGAAEVAATKTELGFDPEAHFAIDDEVIAHTRSLAERNAQKKAAWQVKFDEWAAANPENKALFDRLNSRELPAGYADELPTWDADEKGVATRKASEAALQALGKTLPELWGGSADLAGSNNTVIKGSPSFGPESISTETWSAEPYGRNLHFGIREHAMGSILNGISLHGGTRPYGGTFLIFSDYMRPAVRLAALMETDAYYVWTHDSIGLGEDGPTHQPVETLAALRAIPGLSVLRPADANETAQAWAAALEYKEGPKGLALTRQNVPVLEGTKEKAAEGVRRGGYVLVEGSKETPDVILMGSGSEVQLAVNAAKALEAEGVAARVVSVPCMDWFQEQDAEYIESVLPAAVTARVSVEAGIAMPWYRFLGTQGRAVSLEHFGASADYQTLFEKFGITTDAVVAAAKDSING

SEQ ID NO: 13 - DNA, 2103 bp, synthetic construct
  source 1..2103: mol_type = other DNA
ttgaccaccttgacgctgtcacctgaacttcaggcgctcactgtacgcaattacccctctgattggtccgatgtggacaccaaggctgtagacactgttcgtgtcctcgctgcagacgctgtagaaaactgtggctccggccacccaggcaccgcaatgagcctggctccccttgcatacaccttgtaccagcgggttatgaacgtagatccacaggacaccaactgggcaggccgtgaccgcttcgttctttcttgtggccactcctctttgacccagtacatccagctttacttgggtggattcggccttgagatggatgacctgaaggctctgcgcacctgggattccttgaccccaggacaccctgagtaccgccacaccaagggcgttgagatcaccactggccctcttggccagggtcttgcatctgcagttggtatggccatggctgctcgtcgtgagcgtggcctattcgacccaaccgctgctgagggcgaatccccattcgaccaccacatctacgtcattgcttctgatggtgacctgcaggaaggtgtcacctctgaggcatcctccatcgctggcacccagcagctgggcaacctcatcgtgttctgggatgacaaccgcatctccatcgaagacaacactgagatcgctttcaacgaggacgttgttgctcgttacaaggcttacggctggcagaccattgaggttgaggctggcgaggacgttgcagcaatcgaagctgcagtggctgaggctaagaaggacaccaagcgacctaccttcatccgcgttcgcaccatcatcggcttcccagctccaactatgatgaacaccggtgctgtgcacggtgctgctcttggcgcagctgaggttgcagcaaccaagactgagcttggattcgatcctgaggctcacttcgcgatcgacgatgaggttatcgctcacacccgctccctcgcagagcgccaggcacagaagaaggctgcatggcaggtcaagttcgatgagtgggcagctgccaaccctgagaacaaggctctgttcgatcgcctgaactcccgtgagcttccagcgggctacgctgacgagctcccaacatgggatgcagatgagaagggcgtcgcaactcgtaaggcttccgaggctgcacttcaggcactgggcaagacccttcctgagctgtggggcggttccgctgacctcgcaggttccaacaacaccgtgatcaagggctccccttccttcggccctgagtccatctccaccgagacctggtctgctgagccttacggccgtaacctgcacttcggtatccgtgagcacgctatgggatccatcctcaacggcatttccctccacggtggcacccgcccatacggcggaaccttcctcatcttctccgactacatgcgtcctgcagttcgtcttgcagctctcatggagaccgacgcttactacgtctggacccacgactccatcggtctgggcgaagatggcccaacccaccagcctgttgaaaccttggctgcactgcgcgccatcccaggtctgtccgtcctgcgtcctgcagatgcgaacgagaccgcccaggcttgggctgcagcacttgagtacaaggaaggccctaagggtcttgcactgacccgccagaacgttcctgttctggaaggcaccaaggagaaggctgctgaaggcgttcgccgcggtggctacgtcctggttgagggttccaaggaaaccccagatgtgatcctcatgggctccggctccgaggttcagcttgcagttaacgctgcgaaggctctggaagctgagggcgttgcagctcgcgttgtttccgttccttgcatggattggttccaggagcaggacgcagagtacatcgagtccgttctgcctgcagctgtgaccgctcgtgtgtctgttgaagctggcatcgcaatgccttggtaccgcttcttgggcacccagggccgtgctgtctcccttgagcacttcggtgcttctgcggattaccagaccctgtttgagaagttcggcatcaccaccgatgcagtcgtggcagcggccaaggactccattaacggttaa

SEQ ID NO: 14 - protein, 700 aa, synthetic construct
MTTLTLSPELQALTVRNYPSDWSDVDTKAVDTVRVLAADAVENCGSGHPGTAMSLAPLAYTLYQRVMNVDPQDTNWAGRDRFVLSCGHSSLTQYIQLYLGGFGLEMDDLKALRTWDSLTPGHPEYRHTKGVEITTGPLGQGLASAVGMAMAARRERGLFDPTAAEGESPFDHHIYVIASDGDLQEGVTSEASSIAGTQQLGNLIVFWDDNRISIEDNTEIAFNEDVVARYKAYGWQTIEVEAGEDVAAIEAAVAEAKKDTKRPTFIRVRTIIGFPAPTMMNTGAVHGAALGAAEVAATKTELGFDPEAHFAIDDEVIAHTRSLAERQAQKKAAWQVKFDEWAAANPENKALFDRLNSRELPAGYADELPTWDADEKGVATRKASEAALQALGKTLPELWGGSADLAGSNNTVIKGSPSFGPESISTETWSAEPYGRNLHFGIREHAMGSILNGISLHGGTRPYGGTFLIFSDYMRPAVRLAALMETDAYYVWTHDSIGLGEDGPTHQPVETLAALRAIPGLSVLRPADANETAQAWAAALEYKEGPKGLALTRQNVPVLEGTKEKAAEGVRRGGYVLVEGSKETPDVILMGSGSEVQLAVNAAKALEAEGVAARVVSVPCMDWFQEQDAEYIESVLPAAVTARVSVEAGIAMPWYRFLGTQGRAVSLEHFGASADYQTLFEKFGITTDAVVAAAKDSING

SEQ ID NO: 15 - DNA, 2689 bp, synthetic construct
  source 1..2689: mol_type = other DNA
cagaataattaagcttgcatgcctgcaggtcgacttcacagcggacgatttcaggccctcgtagctcgagagtttgaaggggtccgattcgttccgttcgtgacgctttgtgaggttttttgacgttgcaccgtattgcttgccgaacatttttcttttcctttcggtttttcgagaattttcacctacaaaagcccacgtcacagctcccagacttaagattgatcacacctttgacacatttgaaccacagttggttataaaatgggttcaacatcactatggttagaggtgttgacgggtcagattaagcaaagactactttcggggtagatcacctttgccaaatttgaaccaattaacctaagtcgtagatctgatcatcggatctaacgaaaacgaaccaaaactttggtcccggtttaacccaggaaggattgaccaccttgacgctgtcacctgaacttcaggcgctcactgtacgcaattacccctctgattggtccgatgtggacaccaaggctgtagacactgttcgtgtcctcgctgcagacgctgtagaaaactgtggctccggccacccaggcaccgcaatgagcctggctccccttgcatacaccttgtaccagcgggttatgaacgtagatccacaggacaccaactgggcaggccgtgaccgcttcgttctttcttgtggccactcctctttgacccagtacatccagctttacttgggtggattcggccttgagatggatgacctgaaggctctgcgcacctgggattccttgaccccaggacaccctgagtaccgccacaccaagggcgttgagatcaccactggccctcttggccagggtcttgcatctgcagttggtatggccatggctgctcgtcgtgagcgtggcctattcgacccaaccgctgctgagggcgaatccccattcgaccaccacatctacgtcattgcttctgatggtgacctgcaggaaggtgtcacctctgaggcatcctccatcgctggcacccagcagctgggcaacctcatcgtgttctgggatgacaaccgcatctccatcgaagacaacactgagatcgctttcaacgaggacgttgttgctcgttacaaggcttacggctggcagaccattgaggttgaggctggcgaggacgttgcagcaatcgaagctgcagtggctgaggctaagaaggacaccaagcgacctaccttcatccgcgttcgcaccatcatcggcttcccagctccaactatgatgaacaccggtgctgtgcacggtgctgctcttggcgcagctgaggttgcagcaaccaagactgagcttggattcgatcctgaggctcacttcgcgatcgacgatgaggttatcgctcacacccgctccctcgcagagcgcgctgcacagaagaaggctgcatggcaggtcaagttcgatgagtgggcagctgccaaccctgagaacaaggctctgttcgatcgcctgaactcccgtgagcttccagcgggctacgctgacgagctcccaacatgggatgcagatgagaagggcgtcgcaactcgtaaggcttccgaggctgcacttcaggcactgggcaagacccttcctgagctgtggggcggttccgctgacctcgcaggttccaacaacaccgtgatcaagggctccccttccttcggccctgagtccatctccaccgagacctggtctgctgagccttacggccgtaacctgcacttcggtatccgtgagcacgctatgggatccatcctcaacggcatttccctccacggtggcacccgcccatacggcggaaccttcctcatcttctccgactacatgcgtcctgcagttcgtcttgcagctctcatggagaccgacgcttactacgtctggacccacgactccatcggtctgggcgaagatggcccaacccaccagcctgttgaaaccttggctgcactgcgcgccatcccaggtctgtccgtcctgcgtcctgcagatgcgaacgagaccgcccaggcttgggctgcagcacttgagtacaaggaaggccctaagggtcttgcactgacccgccagaacgttcctgttctggaaggcaccaaggagaaggctgctgaaggcgttcgccgcggtggctacgtcctggttgagggttccaaggaaaccccagatgtgatcctcatgggctccggctccgaggttcagcttgcagttaacgctgcgaaggctctggaagctgagggcgttgcagctcgcgttgtttccgttccttgcatggattggttccaggagcaggacgcagagtacatcgagtccgttctgcctgcagctgtgaccgctcgtgtgtctgttgaagctggcatcgcaatgccttggtaccgcttcttgggcacccagggccgtgctgtctcccttgagcacttcggtgcttctgcggattaccagaccctgtttgagaagttcggcatcaccaccgatgcagtcgtggcagcggccaaggactccattaacggttaattgccctgctgtttttagcttcaacccggggcaatatgattctccggaattttattgccccgggttgttgttgttaatcggtacaaagggtcttaagcacatcccttacttgcctggtaccgagctcgaattcagcttggctgttttgg

SEQ ID NO: 16 - DNA, 2621 bp, synthetic construct
  source 1..2621: mol_type = other DNA
ttcacagcggacgatttcaggccctcgtagctcgagagtttgaaggggtccgattcgttccgttcgtgacgctttgtgaggttttttgacgttgcaccgtattgcttgccgaacatttttcttttcctttcggtttttcgagaattttcacctacaaaagcccacgtcacagctcccagacttaagattgatcacacctttgacacatttgaaccacagttggttataaaatgggttcaacatcactatggttagaggtgttgacgggtcagattaagcaaagactactttcggggtagatcacctttgccaaatttgaaccaattaacctaagtcgtagatctgatcatcggatctaacgaaaacgaaccaaaactttggtcccggtttaacccaggaaggattgaccaccttgacgctgtcacctgaacttcaggcgctcactgtacgcaattacccctctgattggtccgatgtggacaccaaggctgtagacactgttcgtgtcctcgctgcagacgctgtagaaaactgtggctccggccacccaggcaccgcaatgagcctggctccccttgcatacaccttgtaccagcgggttatgaacgtagatccacaggacaccaactgggcaggccgtgaccgcttcgttctttcttgtggccactcctctttgacccagtacatccagctttacttgggtggattcggccttgagatggatgacctgaaggctctgcgcacctgggattccttgaccccaggacaccctgagtaccgccacaccaagggcgttgagatcaccactggccctcttggccagggtcttgcatctgcagttggtatggccatggctgctcgtcgtgagcgtggcctattcgacccaaccgctgctgagggcgaatccccattcgaccaccacatctacgtcattgcttctgatggtgacctgcaggaaggtgtcacctctgaggcatcctccatcgctggcacccagcagctgggcaacctcatcgtgttctgggatgacaaccgcatctccatcgaagacaacactgagatcgctttcaacgaggacgttgttgctcgttacaaggcttacggctggcagaccattgaggttgaggctggcgaggacgttgcagcaatcgaagctgcagtggctgaggctaagaaggacaccaagcgacctaccttcatccgcgttcgcaccatcatcggcttcccagctccaactatgatgaacaccggtgctgtgcacggtgctgctcttggcgcagctgaggttgcagcaaccaagactgagcttggattcgatcctgaggctcacttcgcgatcgacgatgaggttatcgctcacacccgctccctcgcagagcgcgctgcacagaagaaggctgcatggcaggtcaagttcgatgagtgggcagctgccaaccctgagaacaaggctctgttcgatcgcctgaactcccgtgagcttccagcgggctacgctgacgagctcccaacatgggatgcagatgagaagggcgtcgcaactcgtaaggcttccgaggctgcacttcaggcactgggcaagacccttcctgagctgtggggcggttccgctgacctcgcaggttccaacaacaccgtgatcaagggctccccttccttcggccctgagtccatctccaccgagacctggtctgctgagccttacggccgtaacctgcacttcggtatccgtgagcacgctatgggatccatcctcaacggcatttccctccacggtggcacccgcccatacggcggaaccttcctcatcttctccgactacatgcgtcctgcagttcgtcttgcagctctcatggagaccgacgcttactacgtctggacccacgactccatcggtctgggcgaagatggcccaacccaccagcctgttgaaaccttggctgcactgcgcgccatcccaggtctgtccgtcctgcgtcctgcagatgcgaacgagaccgcccaggcttgggctgcagcacttgagtacaaggaaggccctaagggtcttgcactgacccgccagaacgttcctgttctggaaggcaccaaggagaaggctgctgaaggcgttcgccgcggtggctacgtcctggttgagggttccaaggaaaccccagatgtgatcctcatgggctccggctccgaggttcagcttgcagttaacgctgcgaaggctctggaagctgagggcgttgcagctcgcgttgtttccgttccttgcatggattggttccaggagcaggacgcagagtacatcgagtccgttctgcctgcagctgtgaccgctcgtgtgtctgttgaagctggcatcgcaatgccttggtaccgcttcttgggcacccagggccgtgctgtctcccttgagcacttcggtgcttctgcggattaccagaccctgtttgagaagttcggcatcaccaccgatgcagtcgtggcagcggccaaggactccattaacggttaattgccctgctgtttttagcttcaacccggggcaatatgattctccggaattttattgccccgggttgttgttgttaatcggtacaaagggtcttaagcacatcccttacttgcct

SEQ ID NO: 17 - DNA, 2621 bp, synthetic construct
  source 1..2621: mol_type = other DNA
ttcacagcggacgatttcaggccctcgtagctcgagagtttgaaggggtccgattcgttccgttcgtgacgctttgtgaggttttttgacgttgcaccgtattgcttgccgaacatttttcttttcctttcggtttttcgagaattttcacctacaaaagcccacgtcacagctcccagacttaagattgatcacacctttgacacatttgaaccacagttggttataaaatgggttcaacatcactatggttagaggtgttgacgggtcagattaagcaaagactactttcggggtagatcacctttgccaaatttgaaccaattaacctaagtcgtagatctgatcatcggatctaacgaaaacgaaccaaaactttggtcccggtttaacccaggaaggattgaccaccttgacgctgtcacctgaacttcaggcgctcactgtacgcaattacccctctgattggtccgatgtggacaccaaggctgtagacactgttcgtgtcctcgctgcagacgctgtagaaaactgtggctccggccacccaggcaccgcaatgagcctggctccccttgcatacaccttgtaccagcgggttatgaacgtagatccacaggacaccaactgggcaggccgtgaccgcttcgttctttcttgtggccactcctctttgacccagtacatccagctttacttgggtggattcggccttgagatggatgacctgaaggctctgcgcacctgggattccttgaccccaggacaccctgagtaccgccacaccaagggcgttgagatcaccactggccctcttggccagggtcttgcatctgcagttggtatggccatggctgctcgtcgtgagcgtggcctattcgacccaaccgctgctgagggcgaatccccattcgaccaccacatctacgtcattgcttctgatggtgacctgcaggaaggtgtcacctctgaggcatcctccatcgctggcacccagcagctgggcaacctcatcgtgttctgggatgacaaccgcatctccatcgaagacaacactgagatcgctttcaacgaggacgttgttgctcgttacaaggcttacggctggcagaccattgaggttgaggctggcgaggacgttgcagcaatcgaagctgcagtggctgaggctaagaaggacaccaagcgacctaccttcatccgcgttcgcaccatcatcggcttcccagctccaactatgatgaacaccggtgctgtgcacggtgctgctcttggcgcagctgaggttgcagcaaccaagactgagcttggattcgatcctgaggctcacttcgcgatcgacgatgaggttatcgctcacacccgctccctcgcagagcgcactgcacagaagaaggctgcatggcaggtcaagttcgatgagtgggcagctgccaaccctgagaacaaggctctgttcgatcgcctgaactcccgtgagcttccagcgggctacgctgacgagctcccaacatgggatgcagatgagaagggcgtcgcaactcgtaaggcttccgaggctgcacttcaggcactgggcaagacccttcctgagctgtggggcggttccgctgacctcgcaggttccaacaacaccgtgatcaagggctccccttccttcggccctgagtccatctccaccgagacctggtctgctgagccttacggccgtaacctgcacttcggtatccgtgagcacgctatgggatccatcctcaacggcatttccctccacggtggcacccgcccatacggcggaaccttcctcatcttctccgactacatgcgtcctgcagttcgtcttgcagctctcatggagaccgacgcttactacgtctggacccacgactccatcggtctgggcgaagatggcccaacccaccagcctgttgaaaccttggctgcactgcgcgccatcccaggtctgtccgtcctgcgtcctgcagatgcgaacgagaccgcccaggcttgggctgcagcacttgagtacaaggaaggccctaagggtcttgcactgacccgccagaacgttcctgttctggaaggcaccaaggagaaggctgctgaaggcgttcgccgcggtggctacgtcctggttgagggttccaaggaaaccccagatgtgatcctcatgggctccggctccgaggttcagcttgcagttaacgctgcgaaggctctggaagctgagggcgttgcagctcgcgttgtttccgttccttgcatggattggttccaggagcaggacgcagagtacatcgagtccgttctgcctgcagctgtgaccgctcgtgtgtctgttgaagctggcatcgcaatgccttggtaccgcttcttgggcacccagggccgtgctgtctcccttgagcacttcggtgcttctgcggattaccagaccctgtttgagaagttcggcatcaccaccgatgcagtcgtggcagcggccaaggactccattaacggttaattgccctgctgtttttagcttcaacccggggcaatatgattctccggaattttattgccccgggttgttgttgttaatcggtacaaagggtcttaagcacatcccttacttgcct

SEQ ID NO: 18 - DNA, 52 bp, Artificial sequence
  source 1..52: mol_type = other DNA
cagaataattaagcttgcatgcctgcaggtcgacttcacagcggacgatttc

SEQ ID NO: 19 - DNA, 53 bp, Artificial sequence
  source 1..53: mol_type = other DNA
ccaaaacagccaagctgaattcgagctcggtaccaggcaagtaagggatgtgc

SEQ ID NO: 20 - DNA, 32 bp, Artificial sequence
  source 1..32: mol_type = other DNA
ccatgcagccttcttctgtgcagagcgctctg

SEQ ID NO: 21 - DNA, 32 bp, Artificial sequence
  source 1..32: mol_type = other DNA
cagagcgctctgcacagaagaaggctgcatgg

SEQ ID NO: 22 - DNA, 32 bp, Artificial sequence
  source 1..32: mol_type = other DNA
ccatgcagccttcttctgtgcacagcgctctg

SEQ ID NO: 23 - DNA, 32 bp, Artificial sequence
  source 1..32: mol_type = other DNA
cagagcgctgtgcacagaagaaggctgcatgg

SEQ ID NO: 24 - DNA, 32 bp, Artificial sequence
  source 1..32: mol_type = other DNA
ccatgcagccttcttctgtgcagggcgctctg

SEQ ID NO: 25 - DNA, 32 bp, Artificial sequence
  source 1..32: mol_type = other DNA
cagagcgccctgcacagaagaaggctgcatgg

SEQ ID NO: 26 - DNA, 32 bp, Artificial sequence
  source 1..32: mol_type = other DNA
ccatgcagccttcttctgtgcattgcgctctg

SEQ ID NO: 27 - DNA, 32 bp, Artificial sequence
  source 1..32: mol_type = other DNA
cagagcgcaatgcacagaagaaggctgcatgg

SEQ ID NO: 28 - DNA, 32 bp, Artificial sequence
  source 1..32: mol_type = other DNA
ccatgcagccttcttctgtgcctggcgctctg

SEQ ID NO: 29 - DNA, 32 bp, Artificial sequence
  source 1..32: mol_type = other DNA
cagagcgccaggcacagaagaaggctgcatgg

SEQ ID NO: 30 - DNA, 54 bp, Artificial sequence
  source 1..54: mol_type = other DNA
cagtgccaagcttgcatgcctgcaggtcgactctagcgtcattgcttctgatgg

SEQ ID NO: 31 - DNA, 32 bp, Artificial sequence
  source 1..32: mol_type = other DNA
ccatgcagccttcttctgtgcagtgcgctctg

SEQ ID NO: 32 - DNA, 32 bp, Artificial sequence
  source 1..32: mol_type = other DNA
cagagcgcactgcacagaagaaggctgcatgg

SEQ ID NO: 33 - DNA, 59 bp, Artificial sequence
  source 1..59: mol_type = other DNA
cagctatgaccatgattacgaattcgagctcggtaccccggagaagatgaggaaggttc

SEQ ID NO: 34 - DNA, 55 bp, Artificial sequence
  source 1..55: mol_type = other DNA
cagtgccaagcttgcatgcctgcaggtcgactctagaatgcgttctggactgagg

SEQ ID NO: 35 - DNA, 36 bp, Artificial sequence
  source 1..36: mol_type = other DNA
gaaatcgtccgctgtgaagtgcaccgagaacagatg

SEQ ID NO: 36 - DNA, 36 bp, Artificial sequence
  source 1..36: mol_type = other DNA
catctgttctcggtgcacttcacagcggacgatttc

SEQ ID NO: 37 - DNA, 38 bp, Artificial sequence
  source 1..38: mol_type = other DNA
gatttaattgcgccatctgaggcaagtaagggatgtgc

SEQ ID NO: 38 - DNA, 38 bp, Artificial sequence
  source 1..38: mol_type = other DNA
gcacatcccttacttgcctcagatggcgcaattaaatc

SEQ ID NO: 39 - DNA, 60 bp, Artificial sequence
  source 1..60: mol_type = other DNA
cagctatgaccatgattacgaattcgagctcggtacccgctatgacaccttcaacggatc

SEQ ID NO: 40 - DNA, 18 bp, Artificial sequence
  source 1..18: mol_type = other DNA
tgtaaaacgacggccagt

SEQ ID NO: 41 - DNA, 18 bp, Artificial sequence
  source 1..18: mol_type = other DNA
caggaaacagctatgacc

SEQ ID NO: 42 - DNA, 19 bp, Artificial sequence
  source 1..19: mol_type = other DNA
tccaaggaagatacacgcc

SEQ ID NO: 43 - DNA, 19 bp, Artificial sequence
  source 1..19: mol_type = other DNA
gccacaagaaagaacgaag

SEQ ID NO: 44 - DNA, 18 bp, Artificial sequence
  source 1..18: mol_type = other DNA
catcctcaacggcatttc

SEQ ID NO: 45 - DNA, 18 bp, Artificial sequence
  source 1..18: mol_type = other DNA
tggtcgttggaatcttgc

SEQ ID NO: 46 - DNA, 57 bp, Artificial sequence
  source 1..57: mol_type = other DNA
cagtgccaagcttgcatgcctgcaggtcgactctagggaaatagatgggtgtagacg

SEQ ID NO: 47 - DNA, 38 bp, Artificial sequence
  source 1..38: mol_type = other DNA
gcaaggaacggaaacaacgccttcaggtcatccatctc

SEQ ID NO: 48 - DNA, 38 bp, Artificial sequence
  source 1..38: mol_type = other DNA
gagatggatgacctgaaggcgttgtttccgttccttgc

SEQ ID NO: 49 - DNA, 56 bp, Artificial sequence
  source 1..56: mol_type = other DNA
cagctatgaccatgattacgaattcgagctcggtacccatcaacctttgcccacag